European Patent Application EP 4 534 699 A1, published April 9, 2025. Title: 一种宫颈细胞基因甲基化检测试剂盒及其检测方法. Applicant: 青岛瑞思德医学检验实验室有限公司. Application CN. The sequence listing filed with the application follows.

SEQUENCE LISTING (12 sequences)

SEQ ID NO: 1 - DNA, 20 bp, Homo sapiens
  source 1..20: mol_type = genomic DNA
tcggtttttattggtcgcgg

SEQ ID NO: 2 - DNA, 18 bp, Homo sapiens
  source 1..18: mol_type = genomic DNA
tacctcgaaacaaaacgc

SEQ ID NO: 3 - DNA, 14 bp, Homo sapiens
  source 1..14: mol_type = genomic DNA
accgcgaaaccaac

SEQ ID NO: 4 - DNA, 30 bp, Homo sapiens
  source 1..30: mol_type = genomic DNA
tcgacgttgtagtttttcggttagacgaat

SEQ ID NO: 5 - DNA, 21 bp, Homo sapiens
  source 1..21: mol_type = genomic DNA
tacccctccaaaacctcccac

SEQ ID NO: 6 - DNA, 26 bp, Homo sapiens
  source 1..26: mol_type = genomic DNA
cccgaccccaacccaaataacttcat

SEQ ID NO: 7 - DNA, 16 bp, Homo sapiens
  source 1..16: mol_type = genomic DNA
gtttcgcgtcgcgttt

SEQ ID NO: 8 - DNA, 16 bp, Homo sapiens
  source 1..16: mol_type = genomic DNA
acgacgacgaaccacc

SEQ ID NO: 9 - DNA, 13 bp, Homo sapiens
  source 1..13: mol_type = genomic DNA
cgcgccctaaact

SEQ ID NO: 10 - DNA, 16 bp, Homo sapiens
  source 1..16: mol_type = genomic DNA
taggatttttatttag

SEQ ID NO: 11 - DNA, 16 bp, Homo sapiens
  source 1..16: mol_type = genomic DNA
tgtgaatttttgttat

SEQ ID NO: 12 - DNA, 15 bp, Homo sapiens
  source 1..15: mol_type = genomic DNA
ttttaagggaggagt